European Patent Application EP 4 123 307 A1, published January 25, 2023. Title: Methods for structure determination and drug design using Salipro particles. Applicant: Salipro Biotech AB. The sequence listing filed with the application follows.

SEQUENCE LISTING (51 sequences)

SEQ ID NO: 1 - protein, 81 aa, Homo sapiens
SLPCDICKDVVTAAGDMLKDNATEEEILVYLEKTCDWLPKPNMSASCKEIVDSYLPVILDIIKGEMSRPGEVCSALNLCES

SEQ ID NO: 2 - protein, 79 aa, Homo sapiens
GDVCQDCIQMVTDIQTAVRTNSTFVQALVEHVKEECDRLGPGMADICKNYISQYSEIAIQMMMHMQPKEICALVGFCDE

SEQ ID NO: 3 - protein, 80 aa, Homo sapiens
DVYCEVCEFLVKEVTKLIDNNKTEKEILDAFDKMCSKLPKSLSEECQEVVDTYGSSILSILLEEVSPELVCSMLHLCSGT

SEQ ID NO: 4 - protein, 78 aa, Homo sapiens
GFCEVCKKLVGYLDRNLEKNSTKQEILAALEKGCSFLPDPYQKQCDQFVAEYEPVLIEILVEVMDPSFVCLKIGACPS

SEQ ID NO: 5 - protein, 145 aa, Homo sapiens
MATWALLLLAAMLLGNPGLVFSRLSPEYYDLARAHLRDEEKSCPCLAQEGPQGDLLTKTQELGRDYRTCLTIVQKLKKMVDKPTQRSVSNAATRVCRTGRSRWRDVCRNFMRRYQSRVTQGLVAGETAQQICEDLRLCIPSTGPL

SEQ ID NO: 6 - protein, 129 aa, Sus scrofa
PGLAFSGLTPEHSALARAHPCDGEQFCQNLAPEDPQGDQLLQREELGLICESCRKIIQKLEDMVGPQPNEDTVTQAASRVCDKMKILRGVCKKIMRTFLRRISKDILTGKKPQAICVDIKICKEKTGLI

SEQ ID NO: 7 - protein, 77 aa, Entamoeba histolytica
IPVLCPVCTSLVGKLIDLVLGGAVDKVTDYLETLCAKADGLVETLCTKIVSYGIDKLIEKILEGGSAKLICGLIHAC

SEQ ID NO: 8 - protein, 75 aa, Entamoeba dispar
VVCPVCTSLVGKLIDFVIGGAVDKATDYLETLCAKADGVIETVCSKIVSYGIDKLIEKIIEGGSAKLICGLIHAC

SEQ ID NO: 9 - protein, 77 aa, Entamoeba histolytica
GAILCNLCKDTVKLVENLLTVDGAQAVRQYIDNLCGKASGFLGTLCEKILSFGVDELVKLIENHVDPVVVCEKIHAC

SEQ ID NO: 10 - protein, 75 aa, Entamoeba dispar
GLCNLCKDTVNLIENLLTVDGAQAVRQYIDNLCAKADGFLGTLCNKILSFGVDELVKLIENHVDPVVICEKIHAC

SEQ ID NO: 11 - protein, 77 aa, Entamoeba histolytica
GEILCNLCTGLINTLENLLTTKGADKVKDYISSLCNKASGFIATLCTKVLDFGIDKLIQLIEDKVDANAICAKIHAC

SEQ ID NO: 12 - protein, 75 aa, Entamoeba dispar
IVCNLCTGLINTLENLLTTKGADKVKDYIDSLCNKASGFIATLCTKVLDFGVDKLIQLIEDKVDANAICAKIHAC

SEQ ID NO: 13 - protein, 83 aa, Sus scrofa
GLICESCRKIIQKLEDMVGPQPNEDTVTQAASRVCDKMKILRGVCKKIMRTFLRRISKDILTGKKPQAICVDIKICKEKTGLI

SEQ ID NO: 14 - protein, 78 aa, Sus scrofa
GYFCESCRKIIQKLEDMVGPQPNEDTVTQAASQVCDKLKILRGLCKKIMRSFLRRISWDILTGKKPQAICVDIKICKE

SEQ ID NO: 15 - protein, 83 aa, Equus caballus
GIACWSCRKILQKLEDLVGEQPNEATINEAASRVCRNLGLLRGACKKIMRTCLRLISRDILAGKKPQEVCVDIKLCKHKAGLI

SEQ ID NO: 16 - protein, 84 aa, Bos taurus
GLLCGSCQRIIQHLMDKLGDQPDENTVIEAASKVCGKMGPLKGLCKSITKRFLRRIAADITAGKTSRVVCEDIKMCKSKPVGFI

SEQ ID NO: 17 - protein, 81 aa, Fasciola hepatica
EEPHLDISLCESCTNTVNLVKRLLQNSVVETHIRYLVKYLCKGAGSSQDACIKFIQYEVDGAVGYLIQHNATDICHVIRLC

SEQ ID NO: 18 - protein, 83 aa, Homo sapiens
GRDYRTCLTIVQKLKKMVDKPTQTSVSNAATRVCRTGRSRWRDVCRNFMRRYQSRVIQGLVAGETAQQICEDLRLCIPSTGPL

SEQ ID NO: 19 - protein, 83 aa, Naegleria fowleri
SGICNMCQLLVTQVENWVESNDTIMTLEKKLEQVCSVIPGQYSALCTYAVEQYLPIFIHQVEKQFPALTICQDVHLCSSAQAA

SEQ ID NO: 20 - protein, 73 aa, Clonorchis sinensis
CKHCKTLVGRIQDCWQKGRAKSFVEKTLIFLCKLTGHSEEQCTEHAEEFMKHLDDWITGKTPEELCRSLHMCK

SEQ ID NO: 21 - protein, 83 aa, Naegleria fowleri
PSEFCDVCKYAVQQVDQLALQNEAAIQNALLAACQQLGDNQFGKICNTVVLVYGNELVNALVTYENPTRVCSEQLPLCPKNNT

SEQ ID NO: 22 - protein, 88 aa, Caenorhabditis elegans
NPANPLNLKKHHGVFCDVCKALVEGGEKVGDDDLDAWLDVNIGTLCWTMLLPLHHECEEELKKVKKELKKDIENKDSPDKACKDVDLC

SEQ ID NO: 23 - protein, 83 aa, Homo sapiens
SLPCDICKDVVTAAGDMLKDNATEEEILVYLEKTCDWLPKPNMSASCKEIVDSYLPVILDIIKGEMSRPGEVCSALNLCESLQ

SEQ ID NO: 24 - protein, 83 aa, Bos taurus
SLPCDICKDVITAAGNLLKDNATEQEILMYLERTCDWLPKPNMSASCKEIVDSYLPVILDMIKGQMSHPGEVCSALNLCESLQ

SEQ ID NO: 25 - protein, 83 aa, Mus musculus
SLPCDICKTVVTEAGNLLKDNATQEEILHYLEKTCEWIHDSSLSASCKEVVDSYLPVILDMIKGEMSNPGEVCSALNLCQSLQ

SEQ ID NO: 26 - protein, 83 aa, Gallus gallus
SIPCDLCKELVTVVGKVLKDNGTEDEIRSYLEKTCEFLPDQGLASECKEIVDSYLPVIMDMIKEEFDKPEVVCSALSLCQSLQ

SEQ ID NO: 27 - protein, 83 aa, Danio rerio
TVPCDLCKEVLVVVEQLLKDNVTESELLGYLEKACQLIPDEGLANQCKEIVDNYFPVLMGIIQGELDDPGVVCGALGLCVSQQ

SEQ ID NO: 28 - protein, 83 aa, Xenopus laevis
SMPCDFCKEVVTVLGNYLKDNITQDEIKQYLNKVCDFIPDPGLASTCKQEVSDYFTIVLNLLEQELSNPGVLCSSLGLCTSLQ

SEQ ID NO: 29 - protein, 80 aa, Homo sapiens; identical to SEQ ID NO: 3

SEQ ID NO: 30 - protein, 79 aa, Bos taurus
DIYCEVCEFVVKEVAKLIDNNRTEEEILHALDKVCSKLPTSLAEQCQEVVDTYGRSILSILLDEASPELVCSMLHLCSS

SEQ ID NO: 31 - protein, 79 aa, Mus musculus
VILCQTCQFVMNKFSELIVNNATEELLVKGLSNACGVLPDPARTKCQEVVGTFGPSLLDIFIHEVNPSSLCGVIGLCAA

SEQ ID NO: 32 - protein, 80 aa, Gallus gallus
FSVCEICETMVKEVTGLLESNKTEEEIVHEMEVVCYLLPASVKDQCKDFIEVYGQALIDMLLEATNPEAVCVMLKCCAAN

SEQ ID NO: 33 - protein, 79 aa, Xenopus laevis
NVLCEVCELMVSQLEKLLDNNRTRENIKHGLEKVCKLLPSQYTQKCEDMIEEYSDALIELLEQEANPQAICTALGYCSG

SEQ ID NO: 34 - protein, 79 aa, Danio rerio
SPQCAICEYVMKEIENMIQDQTSEAEIVQAVEKVCNILPSTLTAQCKDLIETYGQAIIDLLVQEADPKTVCSFLALCSG

SEQ ID NO: 35 - protein, 81 aa, Homo sapiens
GGFCEVCKKLVGYLDRNLEKNSTKQEILAALEKGCSFLPDPYQKQCDQFVAEYEPVLIEILVEVMDPSFVCLKIGACPSAH

SEQ ID NO: 36 - protein, 81 aa, Bos taurus
GGFCEVCKKLVGYLDRNLEKNSTKEQILAALEKGCSFLPDQYRKQCDQFVTEYEPVLIEILVEVMDPSFVCLKIGACPAAH

SEQ ID NO: 37 - protein, 81 aa, Mus musculus
GGFCEVCKKLVLYLEHNLEKNSTKEEILAALEKGCSFLPDPYQKQCDDFVAEYEPLLLEILVEVMDPGFVCSKIGVCPSAY

SEQ ID NO: 38 - protein, 81 aa, Gallus gallus
GGFCDICKMIVAYADKELEKNATTTEIEALLEKVCHFLPESVSDQCVQFVEQYEPVVVQLLAEMMDPTFVCTKLGVCGAAK

SEQ ID NO: 39 - protein, 81 aa, Danio rerio
GGFCDVCKMAVRYVDGILEQNATQSEIEEAVLKVCSFLPDAVKDECNQLIEQYEPLLVQLLLQTLDPDFVCMKLGACPEAV

SEQ ID NO: 40 - protein, 81 aa, Xenopus laevis
GDYCAVCKMLMRYVDELLEKNATEIRIKAFLGRICNFLPDSMQNECSALVNEYEPLFIQLLLEALDPSFICIKVNLCQNKK

SEQ ID NO: 41 - protein, 79 aa, Homo sapiens; identical to SEQ ID NO: 2

SEQ ID NO: 42 - protein, 79 aa, Bos taurus
GNVCQDCIQLVTDVQEALRTNSTFVEALVDHAKEECDRLGPGMSDMCKNYINQYSEVAIQMVMHMQPKEICVLAGFCDE

SEQ ID NO: 43 - protein, 83 aa, Gallus gallus
EDVCQDCIRLVTDVQEAVRTNATFVKSLVAHAKEECDRLGPGMSDMCKSYISEYSDLAIQMMMHMKDQQPKDICAMVGFCPSV

SEQ ID NO: 44 - protein, 83 aa, Mus musculus
EDVCQDCMKLVSDVQTAVKTNSSFIQGFVDHVKEDCDRLGPGVSDICKNYVDQYSEVCVQMLMHMQDQQPKEICVLAGFCNEV

SEQ ID NO: 45 - protein, 79 aa, Danio rerio
GDVCQDCVTFISDTQDEARVNSSFINTLIAQVENQCELLGPGMSDMCKEYISQYGPLVFQQLMSMQPKDICARAGFCPT

SEQ ID NO: 46 - protein, 79 aa, Xenopus laevis
GDICNDCTKLVSDVQDALRSNSSFSKKLVDHFLQECNLLDPAIAEMCKSYINQYSDIAIQVLLQMQPKQLCGMAGFCDQ

SEQ ID NO: 47 - protein, 74 aa, Glycine max
  Saposin from Soybean (XP_003552303.1)
DVCALCEEYITKALDYLHENKTETEIISILHNTCHQLPSFKQKCVALVDYYVPLFFSEVATIQPGEFCHKVNLC

SEQ ID NO: 48 - protein, 74 aa, Cicer arietinum
  Saposin from chickpea (XP_004506439.1)
DVCSLCEEYTTKALNYIKDNNTQAEIIDGLHNTCYQLLSFKKQCIELVDYYAPLFFSKIALIKPGELCEKFNLC

SEQ ID NO: 49 - protein, 73 aa, Malus x domestica
  Saposin from apple tree (XP_008388327.1)
VCTLCEEFADQALDYLNENKTQTEIIEYLHQTCHQLRSFNQQCVTLVDYYAPLFFLEATSLQPSEFCRKVNLC

SEQ ID NO: 50 - protein, 81 aa, Vicugna pacos
  Saposin A from alpaca
SLPCDICKEVITAAGNMLKDNATEQEILVYLEKTCDWLPKPNMSASCREIVDSYLPVILDMIKGQMSHPEEVCAALNLCES

SEQ ID NO: 51 - protein, 84 aa, Panthera tigris altaica
  Saposin A from Panthera tigris altaica
SLPCDICKDVITAAGDMLKDNATEQEILVYLERTCDWLPNQNLSASCKEMVDTYLPVILDMIKGQMSHPGEVCSALNLCESLQK